European Patent Application EP 4 616 862 A1, published September 17, 2025. Title: Antiviral composition comprising nucleoside analogues derived from nucleic acid or pharmaceutically acceptable salt thereof. Applicant: CJ CheilJedang Corporation. Application WO. The sequence listing filed with the application follows.

SEQUENCE LISTING (28 sequences)

SEQ ID NO: 1 - DNA, 20 bp, synthetic construct
  misc_feature 1..20: note = ASFV specific forward primer
  source 1..20: mol_type = other DNA
agttcggatgtcacaacgct

SEQ ID NO: 2 - DNA, 20 bp, synthetic construct
  misc_feature 1..20: note = ASFV specific reverse primer
  source 1..20: mol_type = other DNA
actggttccctccaccgata

SEQ ID NO: 3 - DNA, 20 bp, synthetic construct
  misc_feature 1..20: note = CSFV specific forward primer
  source 1..20: mol_type = other DNA
ctctggtcagggtgctcaag

SEQ ID NO: 4 - DNA, 20 bp, synthetic construct
  misc_feature 1..20: note = CSFV specific reverse primer
  source 1..20: mol_type = other DNA
gagggactgtgcaaccatca

SEQ ID NO: 5 - DNA, 20 bp, synthetic construct
  misc_feature 1..20: note = LPAIV specific forward primer
  source 1..20: mol_type = other DNA
gctaggcagatggtacaggc

SEQ ID NO: 6 - DNA, 20 bp, synthetic construct
  misc_feature 1..20: note = LPAIV specific reverse primer
  source 1..20: mol_type = other DNA
tgcactcccatccgtttctg

SEQ ID NO: 7 - DNA, 21 bp, synthetic construct
  misc_feature 1..21: note = CCoV specific forward primer
  source 1..21: mol_type = other DNA
tgaaggtgtgccaactggtgt

SEQ ID NO: 8 - DNA, 20 bp, synthetic construct
  misc_feature 1..20: note = CCoV specific reverse primer
  source 1..20: mol_type = other DNA
gcccatcctgtcgcactact

SEQ ID NO: 9 - DNA, 22 bp, synthetic construct
  misc_feature 1..22: note = CAV specific forward primer
  source 1..22: mol_type = other DNA
cgctgaacattactaccttgtc

SEQ ID NO: 10 - DNA, 21 bp, synthetic construct
  misc_feature 1..21: note = CAV specific reverse primer
  source 1..21: mol_type = other DNA
gcagagtctagaacaaatggc

SEQ ID NO: 11 - DNA, 31 bp, synthetic construct
  misc_feature 1..31: note = CDV specific forward primer
  source 1..31: mol_type = other DNA
gcttacttcagactcgggcaagaaatggtta

SEQ ID NO: 12 - DNA, 31 bp, synthetic construct
  misc_feature 1..31: note = CDV specific reverse primer
  source 1..31: mol_type = other DNA
cagtagctcgaattgtccggtcctctgttgt

SEQ ID NO: 13 - DNA, 20 bp, synthetic construct
  misc_feature 1..20: note = FPV specific forward primer
  source 1..20: mol_type = other DNA
agagcattgggcttaccacc

SEQ ID NO: 14 - DNA, 21 bp, synthetic construct
  misc_feature 1..21: note = FPV specific reverse primer
  source 1..21: mol_type = other DNA
ccccatttgagttacaccacg

SEQ ID NO: 15 - DNA, 20 bp, synthetic construct
  misc_feature 1..20: note = FCV specific forward primer
  source 1..20: mol_type = other DNA
gcaaagatccggcttgcctc

SEQ ID NO: 16 - DNA, 20 bp, synthetic construct
  misc_feature 1..20: note = FCV specific reverse primer
  source 1..20: mol_type = other DNA
cgctgttgaccaagtgcagc

SEQ ID NO: 17 - DNA, 22 bp, synthetic construct
  misc_feature 1..22: note = FIPV specific forward primer
  source 1..22: mol_type = other DNA
tggcatcttgctaactggaact

SEQ ID NO: 18 - DNA, 20 bp, synthetic construct
  misc_feature 1..20: note = FIPV specific reverse primer
  source 1..20: mol_type = other DNA
tgccataaacgagccagcta

SEQ ID NO: 19 - DNA, 24 bp, synthetic construct
  misc_feature 1..24: note = FMDV specific forward primer
  source 1..24: mol_type = other DNA
ccgacccctcattcagcagacctc

SEQ ID NO: 20 - DNA, 22 bp, synthetic construct
  misc_feature 1..22: note = FMDV specific reverse primer
  source 1..22: mol_type = other DNA
gagggttcttttccgcgtcgcc

SEQ ID NO: 21 - DNA, 20 bp, synthetic construct
  misc_feature 1..20: note = Forward primer for beta actin
  source 1..20: mol_type = other DNA
gaccaccttcaactcgatca

SEQ ID NO: 22 - DNA, 20 bp, synthetic construct
  misc_feature 1..20: note = Reverse primer for beta actin
  source 1..20: mol_type = other DNA
gtgttggcgtagaggtcctt

SEQ ID NO: 23 - DNA, 20 bp, synthetic construct
  misc_feature 1..20: note = ISG15 forward primer
  source 1..20: mol_type = other DNA
ggtgcaaagcttcagagacc

SEQ ID NO: 24 - DNA, 20 bp, synthetic construct
  misc_feature 1..20: note = ISG15 reverse primer
  source 1..20: mol_type = other DNA
gtcagccagacctcataggc

SEQ ID NO: 25 - DNA, 20 bp, synthetic construct
  misc_feature 1..20: note = Mx1 forward primer
  source 1..20: mol_type = other DNA
agcgcagtgacaccagcgac

SEQ ID NO: 26 - DNA, 20 bp, synthetic construct
  misc_feature 1..20: note = Mx1 reverse primer
  source 1..20: mol_type = other DNA
gcccggttcagcctgggaac

SEQ ID NO: 27 - DNA, 20 bp, synthetic construct
  misc_feature 1..20: note = RNaseL forward primer
  source 1..20: mol_type = other DNA
gccagacctagtggcttctg

SEQ ID NO: 28 - DNA, 20 bp, synthetic construct
  misc_feature 1..20: note = RNaseL reverse primer
  source 1..20: mol_type = other DNA
agaggcccagagagttgtga